European Patent Application EP 4 289 957 A1, published December 13, 2023. Title: Very Long Chain Polyunsaturated Fatty Acid Composition. Applicant: Nippon Suisan Kaisha, Ltd. The sequence listing filed with the application follows.

SEQUENCE LISTING (14 sequences)

SEQ ID NO: 1 - DNA, 39 bp, Artificial Sequence
  Primer
agggaatattaagcttaccatggggctgctggactcaga

SEQ ID NO: 2 - DNA, 45 bp, Artificial Sequence
  Primer
cacactggatcctaggtaccttactctccttttggcttcccgttt

SEQ ID NO: 3 - DNA, 44 bp, Artificial Sequence
  Primer
agggaatattaagcttaccatggaggttgtaacacattttgtga

SEQ ID NO: 4 - DNA, 43 bp, Artificial Sequence
  Primer
cacactggatcctaggtaccctactcccttttcgctcttccct

SEQ ID NO: 5 - DNA, 35 bp, Artificial Sequence
  Primer
gatgatccactagtaggaagtaccttcaaagaatg

SEQ ID NO: 6 - DNA, 42 bp, Artificial Sequence
  Primer
gatccggggttttttttgttttatatttgttgtaaaaagtag

SEQ ID NO: 7 - DNA, 28 bp, Artificial Sequence
  Primer
aaaaaaccccggatcggactactagcag

SEQ ID NO: 8 - DNA, 29 bp, Artificial Sequence
  Primer
tactagtggatcatccccacgcgccctgt

SEQ ID NO: 9 - DNA, 47 bp, Artificial Sequence
  Primer
agggaatattaagcttaccatggatattgtaacacatttagtcaacg

SEQ ID NO: 10 - DNA, 44 bp, Artificial Sequence
  Primer
cacactggatcctaggtaccctagtcccgctttgccctgccctt

SEQ ID NO: 11 - protein, 305 aa, Acanthopagrus schlegelii
MEVVTHFVNDTVEFYKWSLTIADKRVEKWPMMSSPLPTLAISCLYLLFLWAGPRYMQDRQPYTLRKTLIVYNFSMVVLNFYIAKELLLASRAAGYSYLCQPVKYSNDVNEVRIASALWWYYISKGVEFLDTVFFILRKKFNQVSFLHVYHHCTMFILWWIGIKWVPGGQSFFGATINSSIHVLMYGYYGLAALGPQMQKYLWWKKYLTIIQMIQFHVTIGHAGHSLYTGCPFPAWMQWALIGYAVTFIILFANFYYHAYRGKPSSTQKGGKPVANGTSAVTNGHSKAEEVEENGKRQKKGRAKRE

SEQ ID NO: 12 - DNA, 2408 bp, Acanthopagrus schlegelii
acatggggagtggcacctggcttccctcggtgtctaggagattgcaagaagatgatgcggctgagcggactgaatgcataattggcctatcttagtcatagattttcacttgccttgtccagtttcttgccaaattgctgtttaatgtcgaactgtagccggcgcggtgtagaaacttgattagcggtgacggcaggagaagggaagaaggggagaagaaggagaagaggagcggagcggtgactgagagaggagttgggcatcaaattgcaccggatgtcattacacgctcttaaatatcgaggactataatcgagaccaaaggcagagccatggaggttgtaacacattttgtgaatgacactgtagaattttacaaatggagccttactatagcagacaagagggtggagaagtggcccatgatgtcatctcccctccccactctggccatcagctgcctgtacctgctcttcctgtgggcggggccccgatacatgcaggaccgccagccctacacgctcaggaagaccctcatagtctacaacttcagcatggtggtcctcaatttctacatcgccaaagagctcctactagcctctagagcagctgggtacagctacctctgtcaacctgtcaagtactccaatgatgtcaacgaagtcaggatagcatctgctctctggtggtactacatctccaaaggcgtggagttcctggatacagtctttttcatcctcaggaagaagttcaaccaggtcagcttcctccacgtctaccaccactgcaccatgttcatcctctggtggatcggcatcaaatgggtccccggtggacagtcattttttggtgcaaccatcaactcttccatccacgtgctcatgtacggatactacggcctggcagccctgggacctcagatgcagaagtacctctggtggaagaaatacctcaccattatccagatgatccagttccacgtgaccatcggccacgccggccactccctctacacaggctgcccattccccgcctggatgcagtgggctttgatcggctacgctgtcaccttcatcatcctcttcgccaacttctactaccacgcttaccgaggcaaaccttcatccacgcagaagggaggcaagcccgtcgccaacggcacctctgcggtaactaacggtcacagcaaagcggaggaggtggaggaaaatgggaagaggcaaaagaagggaagagcgaaaagggagtaaagaagaaagagggcgtgcttggcgattaacagagagaggacagttgttttaaaaagggccagagatgaagggaggagagggataaacagcgaagttcaaaccagaccggcttcattatccctgcaaataatgtagaaggaggtgatgttggtgaccaacttggaaaggtggaaaagtagcagtgtgtgtgtttgtggatgtgtctgtaagggtttctggatttgaaaggttgtgttggttgtcttccatagcagttttttttttcttttttaaatcaagaaaaagcaaaatgctgaccacgtaggatccgcgctcatctgtccaactggggttttggactgtagtaggaccaaagtatttaaaatgggcctacaagctgctcagcatccattaacttatcaaccaaaattcactcaacttttgtactctggattccagtattattttaactgaaagcttgaatagtctttaatatgcttatttattttctagtgctctaaaagagttttaatgaatttaactattaccaacaaaagaacatgcagaagtttataccaaaggtttattttcttggttcgggttttttttcttgttttacgaatatttagcaagttagcaaacaaacaaaaaaaggttacaaatctcacgactgccatctattgtattgaactactttttaattattcacactatctaccaatccaacatgtcatggactttacatttctctgctgtctcaatctgaagtaactgtgcttttttgcacttgcagacattctctttgtgttcattgtgaattaaaatgttggtttaaaacactttgggaggggactgtagttttattttagtctttatgcaaatgtgtgggtatatttgttatgatttctttttgtgggtcctcatgatttatttctttttgctgtgcgatgtagccgaggtgcaagaataagagattgaatttcagctcagtactgtctcactgccatgtaggactgaagggaaacctgacaagagctttttttttattttaaagaaaacaaatggttatttcattgtcttattaagaatcaataaacgacacagcttcgggctgcacatataactgaaataaagacaatgtcagccccccaaaaaaaaaaaaaaaaaaaaaaaaaaaaa

SEQ ID NO: 13 - protein, 314 aa, Clarias gariepinus
MDIVTHLVNDTIEFYKWSLTIADKRVEKWPLMGSPLPTLAISSSYLLFLWLGPKFMRNREAFQLRKTLIVYNFSMVILNFFIFKELFLAARAANYSYLCQPVDYSDDPNEVRVAAALWWYFVSKGVEYLDTVFFILRKKFNHVSFLHVYHHCTMFTLWWIGIKWVAGGQSFFGAHMNAAIHVLMYLYYGLAACGPKIQKYLWWKKYLTIIQMIQFHVTIGHTALSLYTDCPFPKWMHWCLIGYALTFIVLFGNFYYQTYRRQPRREGLSKAGKALSNGASNGMAISNGVSGKMVEKPVVVENGRRKRKGRAKRD

SEQ ID NO: 14 - DNA, 1403 bp, Clarias gariepinus
aaactgtttccactggagcgccgagagagcagcagccacaaacgcactgatgcaaatgtccgtgtaggatgctctgtacatacacccaggacaattaggacgtattttgcagagatggatattgtaacacatttagtcaacgacactatcgaattctacaaatggagtcttaccattgcagacaaacgtgtggaaaaatggcctcttatgggctctcctctccccacactggccatcagctcctcatacctgctcttcctctggctggggccaaagttcatgcggaacagggaggcttttcagctcaggaagaccctaattgtgtacaatttcagcatggttattcttaactttttcatcttcaaagagctcttccttgcagcaagggcagcaaactacagctacctctgccagccagtggactattctgatgaccctaatgaagtcagggttgcagctgctctctggtggtactttgtgtcaaagggggttgaatatctggacacagtgtttttcatccttcgtaaaaagttcaaccatgtcagctttttgcacgtgtatcaccactgcaccatgtttacactgtggtggattggcatcaaatgggttgcaggtggacagtcattttttggtgctcatatgaatgctgcaatccatgttcttatgtatctatattatggactggctgcgtgtggtcccaagatccagaaatacttgtggtggaagaagtacctgacaattatccaaatgatccagttccatgtcactattggtcatactgctctatcgctctacactgactgccccttccctaaatggatgcactggtgtctgattggttatgccctcaccttcattgtcctctttgggaacttttactaccagacatatcgtcgccagccacgccgtgaaggtctgtccaaggctggcaaggcactgtctaatggagcttctaatggaatggcaatcagtaatggagtgagtggcaagatggtggagaagcctgtggtagtggaaaatgggaggaggaagaggaagggcagggcaaagcgggactagagcagatgaaggattgagatgcagaagcaggcatatttgagaaaggatataagagatgggacatttgttaaggagcagtacatttgtaggatgccagggatgaggatatgactgtttggaggaggctcaaaggtcactgtgtgggctttgctaccaccagttagggtggataagattagaaatatttgttaagaacaaacatttggtccttctgtttacagctgtgtttttgctgattttatgcataagcaaccctgtaataagaatgaaatagtcatgattaagggagcctgaattctctatcaaagcatacaattatttaaacaattcctaaaaaaaaaaaa